European Patent Application EP 4 357 354 A1, published April 24, 2024. Title: Epitope peptide of human alpha-synuclein and pharmaceutical composition comprising the peptide. Applicant: Sumitomo Pharma Co., Ltd. The sequence listing filed with the application follows.

SEQUENCE LISTING (26 sequences)

SEQ ID NO: 1 - protein, 9 aa, Artificial Sequence
  p54
KKDQLGKNE

SEQ ID NO: 2 - protein, 9 aa, Artificial Sequence
  p150
EAYEMPSEE

SEQ ID NO: 3 - protein, 10 aa, Artificial Sequence
  p283
EAYEMPSEDG

SEQ ID NO: 4 - protein, 9 aa, Artificial Sequence
  p142
KKDQLGANE

SEQ ID NO: 5 - protein, 10 aa, Artificial Sequence
  p167
KKDQLGKNEE

SEQ ID NO: 6 - protein, 9 aa, Artificial Sequence
  p227
KRDQLGKNE

SEQ ID NO: 7 - protein, 9 aa, Artificial Sequence
  p233
KKDQLGKND

SEQ ID NO: 8 - protein, 9 aa, Artificial Sequence
  p272
KKNQLGKND

SEQ ID NO: 9 - protein, 9 aa, Artificial Sequence
  p273
KKTQLGKND

SEQ ID NO: 10 - protein, 10 aa, Artificial Sequence
  p276
DAYEMPSEEG

SEQ ID NO: 11 - protein, 10 aa, Artificial Sequence
  p277
EAFEMPSEEG

SEQ ID NO: 12 - protein, 8 aa, Artificial Sequence
  DMPVDPDN
DMPVDPDN

SEQ ID NO: 13 - protein, 20 aa, Artificial Sequence
  AJ peptide
ELKLIFLHRLKRLRKRLKRK

SEQ ID NO: 14 - protein, 140 aa, Homo sapiens
MDVFMKGLSKAKEGVVAAAEKTKQGVAEAAGKTKEGVLYVGSKTKEGVVHGVATVAEKTKEQVTNVGGAVVTGVTAVAQKTVEGAGSIAAATGFVKKDQLGKNEEGAPQEGILEDMPVDPDNEAYEMPSEEGYQDYEPEA

SEQ ID NO: 15 - protein, 5 aa, Artificial Sequence
  linker
GGGGS

SEQ ID NO: 16 - protein, 5 aa, Artificial Sequence
  linker
EAAAK

SEQ ID NO: 17 - protein, 5 aa, Artificial Sequence
  linker
DDAKK

SEQ ID NO: 18 - protein, 10 aa, Artificial Sequence
  p242
AAYEMPSEEG

SEQ ID NO: 19 - protein, 10 aa, Artificial Sequence
  p244
EAAEMPSEEG

SEQ ID NO: 20 - protein, 10 aa, Artificial Sequence
  p347
HAFEMPSEEG

SEQ ID NO: 21 - protein, 10 aa, Artificial Sequence
  p361
DAFEMPSEEG

SEQ ID NO: 22 - protein, 9 aa, Artificial Sequence
  p229
KKTQLGKNE

SEQ ID NO: 23 - protein, 9 aa, Artificial Sequence
  p237
KKNQLGKNE

SEQ ID NO: 24 - protein, 9 aa, Artificial Sequence
  p298
KKDELGKDE

SEQ ID NO: 25 - protein, 4 aa, Artificial Sequence
  linker
KKKK

SEQ ID NO: 26 - protein, 6 aa, Artificial Sequence
  linker
PPDPDP